European Patent Application EP 4 249 583 A1, published September 27, 2023. Title: USE OF FATTY ACID ELONGASE GENE AND ESTERASE GENE IN SYNTHESIS OF NERVONIC ACID AND GREASE IN YEAST. Applicant: QINGDAO INSTITUTE OF BIOENERGY AND BIOPROCESS TECHNOLOGY, CHINESE ACADEMY OF SCIENCES ZHEJIANG ZHENYUAN PHARMACEUTICAL CO., LTD. The sequence listing filed with the application follows.

SEQUENCE LISTING (52 sequences)

SEQ ID NO: 1 - DNA, 1563 bp, Malania oleifera
atggcggaagtgagagctgcacgttcaccagaatcagcagggatcaacagcagatcgaacaagcacaacctccccaacttcctcctctccgtcagactgaagtacgtgaagctgggctaccactacttaatctcccacgccatgtacctcttgctcacgccgctcctcgccgccgtcacagctcacctctccaccctcaccctcgacgacttcctccacctctggaaccacctcaaattcaacctggtcaccgtcgtactcggctccaccctcatcgtcttcctcgccaccctctacttcatgagccgcccccgccaggtctacctcttggacttcgcctgctacaagcccgaccccgcccggatatgcagccgcgaagtgttcctaaagcggtcggcgctgacggggacgttctcggcggagaacttggcgttccagaagaagctgatgacgcggtcggggctggggcagaagacgtacttgccggaggcggtgatgcgggtgccgccgaacccgtgcatggcggaggcgaggaaggaggcggagacggtgatgttcggggccatcgacgagctgctggcgaagacgggggtgaaggccaaggatattgggatactggtagtaaactgcagcttgttcaatccgacgccgtcgctttcggcgatggtggtcaaccattacaagctgagggggaacattctgagttataatctgggcgggatggggtgcagcgccgggctaatttccattgaccttgccaagcagcttttgcaggtgcaccccaactcgtacgccctggtagtcagcatggagaacatcaccctgaactggtacttcggcaacaaccgctccatgctcctcccgaactgcctcttccgcatgggcggcgctgccatcctcctctccaaccgcccctccgaccgccgccgctccaagtaccggctcatccacaccgtccgcacccacaagggctccgacgacaagtgctaccgctgcgtcttccagcacgaggacgacgaccgcaacgtcggtgtcgccctctccaaagatctcatggctgtcgctggcgagaccctcaagaccaacatcaccaccctcggccccctcgtcctccctatctccgagcaactcctcttcttcgccaccctcgtcgcccgcaaaatcctcaagatcaaaatcaaaccctacattcccgacttcaagctagccttcgaacatttctgcatccacgccggcggccgcgcggttctcgacgaggtggagaagaacctcgacctctccgaccggcacatggaaccttctagaatgacgctgtacaggttcggcaacacttccagcagctctctgtggtacgagctggcttactcggaggccaaggggaggatccgaaagggtgatcggacgtggcagatcgctttcggatccgggttcaagtgtaacagcgccgtgtggcgggcgctccggaccgtcgatccgtccaaggagaagaacccctggacggacgagattgatgggtttcctgttcatgtgcctgaagaggcaactctggatggaacttcttaa

SEQ ID NO: 2 - DNA, 1674 bp, Malania oleifera
atgctggaactgcaggagtggcctcgacgactgcaaagagatggactgcagcaggcctctgccggagccgtgagaagagttgctgatgaagtggctggagccatggccgatgtgaaaaaacaaaaccccgaccagaacgacgccgtgtctccccatagacaaggccgaaaaatcaactctgccaccctgcccaacttcaagctgtctgtgaagctgaagtacgtgaagctgggctaccactacctgatctctaaggccatgtacgtgttcctgatccccctgctggcctctttctctctgcacttctacaccttcaccgtggacgacctgtctcgagtgtggacccatcacaagttcgacgtgtctaccgtgatcatctgctctggcctgtctatcttcctggccaccgtgtacttcaccacccgacccagaaaagtgtacctgctgaacttctcttgcttcaagcccgagcccgcccgaatttgccctagagaaatgttcatcgaccgatctgtgcgaaccggccgattcaccgaagaaaacctggcttttcagaagaagatcgtggagcgatctggcctgggccagaaaacttatctgcccgaagccgtgctgcgaatcccccctaatccttgtatggccgaagctatgaaggaggccgaaatggtgatgttcggcgccatcgacgaactgctggagaagaccggagtgcgagtgagagagattggcatgctgctggtgaactgctctctgttcaaccccaccccctctcactgcgccactattatgaatcactacaagatgaagggcaacctgctgtgctacaacctgggcggcatgggctgttctgccggacctatcatgatcgacctggccaaacacctgctgcaggtgcaccctaattcttacgccctgattgtgaccatggagaacatcaccctgaactggtacctgggcaacaaccgatctatgctggtgtctaactgcctgttccgaatgggcggcgccgctgtgttactttctaatagattttctgaccgacgacgatctaagtaccagctgatgcacaccgtgcgaacccacaagggcgctgatgattcttgctacgactgcgtgttccagaaggaggacgagaaggacgagatcggcgtgtctctgtctaaggacctgatgatggtggcccgagaggcccttagaactaatattactaccctgggccccctggtgctgcccattactgaacaactgctgttcttcgcctctttcctgggccgaaagatcctgaagatgaacatgaagcagtacctgcccaacttcaagctggccttcaagcacttctgcatccacgccggcggacgagctgtgctggatgaactgcaaaaaaacctggagctgtctgagtggcacatggagccctctcgaatgaccctgtaccgattcggcaacacctcttcttcttctctgtggtacgagctggcctactctgaggccaaaggccgaattaagaagggcgaccgactgtggcagatcgcctttggatctggattcaagtgcaactctgccgtgtggcacgccctgaaaaccatcgatcccgccagagaaaaaaacccctggatggacgagattgacgagttccccgtggacgtgcccaaagtggcttctctgatttcttaa

SEQ ID NO: 3 - DNA, 1539 bp, Malania oleifera
atggctgagcccaagctggacaaacccctgattgccccttctgcttcttctcgactgcccgacttcaagcagggcgtgaaactgaagtacgtgaagctgggctaccactacctggtgacccacgccatgtatctgttcctgtctcccctggccgtgatcaccgtggtgcaactgtctactttctctctgcaggacgtgcacgacctgctgggcaaactgagatataacctgatctctgtgatcctgtgctcttctaccctggtgttcctgtctaccctgtacttcctgacccgaccccgacccgtttatctggtggatttttcttgcttcaagcccgacgacgacgacaagaagtgctcttggcagcgattcatcaagtgctctgagtctatcggcaccaccaccgaggagaacatcgagttccagcgaaagatcatggtgcgatctggcctgggcgagtctacctatttacctcccgctattctgaacattccccctaatccctctatggccgaggccaccgaagaggtgaaaatgatcatgttcggcgccctggaccacctgttcgagaaaacttctgtgaaccccaaggacatctctatcctgatcgtgaactgctctatcttcaaccccaccccctctctgtctgccatggtggtgaatcactacaagctgcgagagaacatccgaacctacaacctgggcggcatgggctgttctgcttctctgatttctatcgacctggccaaggacctgctgcgagtgaattctaactcttacgccctggtggtgtctatggagtctatcaccatgaactggtacttcggcaacgagaagtctatgatcctgtctaactgcctgttccgaatgggcggcgccgctgtgctgctgtctaataaaatgtctgaccgatggcactctaagtacaagctggtgcacaccgtgcgaacccaccgaggatctgatgacaagtgctacacctgcgccacccagcgagaagactctattggcaagatcggcatctctctgtctaaggacctgatggccgtggccggcgatgctctgaaagctaatattactaccctggaccccctggtgctgcctatctctaaacagctgctgttcttcgccaccctggtgggcagaaaatttttcaaggtgaagatgaagccctacatccccgacctgaagctggcctttgaacacttctgcatccacgccggcggccgagctgtgctggatgaactgcaaaaaaacctgcagctgaccgactggcacatcgagccctctagaatgaccctgtaccgattcggcaacatcctgtcttcttctatctggtacgagctggcctacaccgaggccaaaggcagagtgaaaaaaggcgaccgaacttggcagatcaccctgggctctggctttaagtgcaactctgccgtgtgggaggccctgcgaactattaaccctgagaaagaaaagaacccctggatgatcgagatccaccagttccccgtgaacgtgcccaaagtgtctgccatttaa

SEQ ID NO: 4 - DNA, 1539 bp, Malania oleifera
atggctcaaccaaagcttgtcaaacccttgatcgctccatctgcttccccaagacttcctgatttcaaacagggtgtgaaactgaaatatgtgaaactgggctaccattacctcgttactcatgcaatgtacctcttcctaccacctcttgcagtcatcgctgcagtccagctctccacattctcactccaagatgttcatgaccttttggggcagctccggtacaatctcatttcagtgatcctttgctccagcacccttgtctttctatccactctttatttcctcactcgcccccgccctgtttatcttgttgatttctcgtgctttaagcctgatgatgatgataaaaaatgctcgtggcaacgtttcatgaagtgttctgaatcaagaggtacattcactgaggaaaatattgagttccaaaggaaaattatggcaagatctggtattggtgaatcaacttacctgccaccagctgttatgaaaattcctccaaattcgtcaatggcggaagcgagagaagaagccaagatgataatctttggtgttcttgatcgcctctttgagaaaacctcagtgaaaccaaaagatatcagtatcctaattgtcaattgtagcttattcaatcccgtaccttctctatctgcaatggttgttaaccattacaagctaagagggaacacacgtacttataatttgggtgggatgggttgtagtgctggtttgatctcaattgatcttgcaaaagacctacttcgagttcatcccaattcttatgcattggttgtaagcatggaaagcatcactatgaattggtattttgggaatgagagatcaatgatcgtcccgaattgcttgttccgaatgggaggggcagcagttttgctttccaacaagatgtccgaccgatggcattctaagtacaaattggtccacactgtccggactcacaaaggttctgatgataagtgctatacttgtgttacccagcgagaggattccattgggaagattgggatttctttgtcaaaggatctgatggcagttgctggcgatgccctgaaggcaaacatcactacattgggcccccttgtgctaccaatgtctgaacagctactcttctttgcaacattggtcgggaggaaattttttaaggtgaaggtgaagccttacatcccagatttcaagctagcttttgagcatttctgtattcatgctgggggaagagctgtgctagatgaattgcaaaagaacttgcagcttactgattggcatatcgaaccttcaaggatgacactataccgttttggcaacacatcaagtagctctctctggtatgaattggcttataccgaagccaagggaagggtgaagaaaggagatagaacatggcaaatagcatttggttctgggttcaagtgtaacagtgcagtttgggaggctctaagaactatcaaccccgcaaaggagaagaatccatggatgacggagatccaccagttccctataaatgttccgcaagtctcggccatctaa

SEQ ID NO: 5 - DNA, 1962 bp, Malania oleifera
atggccgagcccaagctggacaaacctctgatcgctccctctgcctctcccagactgcctgattttaaacagggcctgaagctgaagtacgtgaagctgggctaccactacctggtgacccacgccatgtacctgttcctgtctcccctggccgtgatcaccgtggttcaactgtctgctttttctctgcaggacgtgcacgacctgctgggccaacttcaatacaatatcatctctgtgatcctgtgctcttctaccctgctgttcctgtctaccctgtacttcctgacccgaccccgacccgtttatctggtggacttttcttgtttcaagcccgacgacgacaacaagtgctcttggcagcgattcatgaagtgctctgagtctatcggcaccttcaccgaggagaacatcgagttccagcgaaagatcatggcccgatctggcctgggcgaatctacttatctgcctcccgctgtgatgaacattccccctaacccctctatggccggcgccagagaagaagctaaaatgatcatgttcggcgccctggaccgactgttcgagaaaacctctgtgaagcccaaggacatctctatcctgatcgtgaactgctctctgttcaaccccgtgccctctctgtctgccatggtggtgaatcactacaagctgcgaggcaacatccgaacctacaacctgggcggcatgggctgttctgccggactgatttctattgacctggccaaggacctgctgcgagtgcatcctaattcttacgccctggtggtgtctatggagtctatcaccaccaactggtacttcggcaacgaccgatctatgatcctgtctaactgcctgatccgaatgggcggcgccgctgttctgctgtctaataaaatgtctgaccgatggcactctaagtacaagctggtgcacaccgtgcgaacccacaagggctctgatgacaagtgctacacctgcgtgacccagcgagaggactctatcggcaaaatcggcatctctctgtctaaggacctgatggccgtggccggcgatgccctgaaagctaatattactaccctgggccctctgatgctgcccatgtctgaacagctgccctttttcgccaccctggtgagacgaaagttcttcaaggtgaaggtgaagccctacatccccgacttcaagctggccttcaagcacttctgcatccacgccggcggacgagctgtgctggatgaattacaaaaaaacctgcagatcaccgactggcacatcgagccctctcgaatgaccctgtaccgattcggcaacaccctgtcttcttctctgtggtacgagctggcctacatcgaggccaaaggcagagtgaaaaagggcgatcgaacttggcagatcgccttcggccctggatttaagtgcaattctgccgtgtgggaggccctgcgaactattaatcctgccaaggagaagaacccctggatgaccgagatcgaccgattccccgaactgatcgtgggctgcggaagaagagattggtctgtggtggctggcgtgcagagaggcgaagctcaacaacaacaactgcaaaagggcggagccgctgtggtgtttaacggcctgcccgaaggagtgctgcaacagcgactgcaacgaagatgctggaagcagctgtgccgaggcctggctcgatctcaagaacttctgctgggactggtgtgttgggctgatggatgctctgcttggtgccgaggcctgctgcaagaaatggccgctagaggatgttgctctgccctgctggaaaagcgactggccagactggctgctgtgctgtgtgctgctgaagaactgggcgctctgttttgctatggaggctctctgggctggctggtgctggctgctgctgttagacgagtgtgttggtgtatgggagatggctgggaacagggcggcagaagataa

SEQ ID NO: 6 - DNA, 1668 bp, Malania oleifera
atgcacgccgccatctctgtgttccaccagttccgacagatccccacctgcatcggccaactgattgaggacttccacctggccctgacctctaccgctgtggatattaactggcgagacgagaaggagccccgaaaggtggaactgggcgctggactgattgatctgaataccatgctgcctgatttcctgcagtctgtgaagctgaagtacgtgaagctgggctacggctactcttgcaaccccgccactattctgactttcctggtggtgctgcccctgtttgtggccactgttgtgcaactgtctggactgagactggcccgagtgtacgaactgtggatgtctcgaggcatccccctggacgctgctacaggaattactggactggctgtgctgctgatcctggtgggagtgtatctggcccgacgatctagacctgtgtacctggtggatttcgcctgctacaagcccgaggacgagcgaaaaatgtctaacgactctttcctgaccatgaccgaggagtctggcgcctttgaggaggagactgtgcaattccaacgacgaattaccaagcgatctggcctgggcgatgagacctatctgccttctggcatcacctctcgaccccctaatctgtgtatgcaggaggcccgatctgaggccgaatctgtgatgttcggcgccctggattctctgttcgacaagaccggcatccgacccgaggatgtgggaatactgatcgtgaattgctctctgttcaaccccaccccctctctgtcttctatgatcgtgaaccactacaagctgcgacccgacatcaagtctatcaacctgggcggcatgggctgctctgccggactgatttctatcgacctggcccgacatctgctgcaggccaatcctaatacttatgccgtggtggtgtctaccgagaacatcaccctgaactggtacttcggcaacgaccgatctatgctgctgtgcaactgcatcttccgaatgggcggcgccgctgtgctgctgtctaataaaacttgggaccgagtgtggtctaagtacgagctggtgcacaccgtgcgaacccacaaaggagctgatgacaattctcacaactgcatctaccagcgagaggacgacaagggcaccgtgggagtgtctctggctagagaactgatggccgtggccggcgatgctcttaaaactaatattaccactctgggcccttctgtgctgcccttttctgagcagttcatgttcttcgtgtctctggtgcgacgaaaggtgatgaaggccaaggtgaagccctacatccccgacttcaagctggccttcgagcacttctgcatccacgccggaggaagagctgtgctggatgaactgcaaaaaaatctgcagctgtctgagtggcacatggagccctctcgaatgaccctgcaccgattcggcaatacctcttcttcttctctgtggtacgagctggcctacaccgaggccaaaggcagagtttctcgaggagatagagtgtggcaaattgccttcggctctggcttcaagtgcaactctgccgtgtggcgagccctgaaagccattcccgctggagaatgtagaggcaatccctgggccgattctgtgcacagataccccgttatgatccccgccgcttaa

SEQ ID NO: 7 - DNA, 1521 bp, Brassica rapa
atgacgtcccgtaacgttaagctcctttaccattacgtcataaccaaccttttcaacctttgcttctttccgttaacggcgatcgtcgccggaaaagcctatcggcttaccatagacgatcttcaccacttatactattcctatctccaacacaacctcataaccatcgctccactctttgccttcaccgttttcggttcggttctctacatcgcaacccggcccaaaccggtttacctcgttgagtactcatgctaccttccaccaacgcattgtagatcaagtatctccaaggtcatggatatcttttatcaagtaagaaaagctgatccttctcggaacggcacgtgcgatgactcgtcgtggcttgacttcttgaggaagattcaagaacgttcaggtctaggcgatgaaactcacgggcccgaggggctgcttcaggtccctccccggaagacttttgcggcggcgcgtgaagagacggagcaagttatcattggtgcgctagaaaatctattcaagaacaccaacgttaaccctaaagatataggtatacttgtggtgaactcaagcatgtttaatccaactccgtcgctctccgcgatggtcgttaacactttcaagctccgaagcaacgtaagaagctttaaccttggtggcatgggttgtagtgccggcgttatagccattgatctagcaaaggacttgttgcatgtccataaaaatacgtatgcccttgtggtgagcacagagaacatcacttataacatttacgctggtgataataggtccatgatggtttcaaattgcttgttccgtgttggtggggccgctattttgctctccaacaagcctggagatcgtagacggtccaagtacgagctagttcacacggttcgaacgcataccggagctgacgacaagtcttttcgttgcgtgcaacaaggagacgatgagaacggcaaaaccggagtgagtttgtccaaggacataaccgatgttgctggtcgaacggttaagaaaaacatagcaacgttgggtccgttgattcttccgttaagcgagaaacttctttttttcgttaccttcatgggcaagaaacttttcaaagataaaatcaaacattactacgtcccggatttcaaacttgctattgaccatttttgtatacatgccggaggcagagccgtgattgatgtgctagagaagaacctagccctagcaccgatcgatgtagaggcatcaagatcaacgttacatagatttggaaacacttcatctagctcaatatggtatgagttggcatacatagaagcaaaaggaaggatgaagaaaggtaataaagtttggcagattgctttagggtcaggctttaagtgtaacagtgcagtttgggtggctctaaacaatgtcaaagcttcgacaaatagtccttgggaacactgcatcgacagatacccggtcaaaattgattctgattcaggtaagtcagagactcgtgtccaaaacggtcggtcctaa

SEQ ID NO: 8 - DNA, 1521 bp, Brassica tournefortii
atgacgtccgttaacgttaagctcatttaccattacgtcataaccaaccttttcaacctttgcttcttcccgttaacggcgatcgtcgccggaaaagcatctcggcttaccatagacgatcttcaccacttatactactcctatctccaacacaacctcataaccattgctccactctttgccttcaccgttttcggttcggttctctacatcgcaacccggcccaaaccggtttaccttgttgagtactcatgctaccttccaccaacgcattgtagatcaagtatctccaaggtcatggatatattttatcaagtgagaaaagctgatccttctcgtaacggcacgtgcgatgactcgtcctggcttgacttcttgaggaagattcaagaacgttcaggtctaggagatgaaactcacggtccagagggactgcttcatgtccctccccggaagacttttgcggcggcgcgtgaagagacggagaaagtaatcatcggtgcgctagaaaatctattcgagaacaccaaagtcaaccctaaagatataggtatacttgtggtgaactcaagcatgtttaatcccactccttcgctctcagcgatggtcgttaatactttcaagctccgaagcaacgtgagaagctttaatctcggtggcatgggctgtagtgccggcgttatagccattgacctggcgaaggacttgttgcatgtccataaaaacacgtatgctcttgtggtgagcaccgagaacatcacttataacatctatgctggtgataataagtccatgatggtttcaaactgcttgttccgtgttggtggggccgctattttgctctccaacaagcctagagatcggagacggtccaagtacgagctagttcacaccgtccgaacgcataccggagctgacgacaagtcttttcgttgcgtgcaacaaggagacgatgagagcggcaaaaccggagtgagtttgtccaaagacataaccgatgtagctggtcgaacggttaagaaaaacatatcaactttgggtccgttgattcttcctttaagcgagaaacttctttttttcgttaccttcatgggcaagaaactcttcaaagacaaaatcaaacattattacgtcccggatttcaaacttgctattgaccatttttgtatacatgccggaggcagagctgtgatcgacgtgctagagaagaacctaggcctagcaccgatcgatgtggaggcatcaagatcaacgttacatagatttgggaacacttcatctagctcaatatggtatgaattggcatacatagaagcaaaaggaaggatgaagaaagggaataaagtttggcagattgctttagggtcagggtttaagtgtaacagtgcggtttgggtggctctacgcaatgtcaaggcttcgagaaaaagtccttgggaacattgcatcgacagatacccagttaaaattgattatgattcagctaagtcagaggttcgtgtccaaaacggtcggtcctaa

SEQ ID NO: 9 - DNA, 1521 bp, Brassica elongata
atgacgtccgttaacgttaagctcctttaccattacgtcataaccaacctcttcaacctttgtttctttccgttaacggcgatcattgccggaaaagcgcatcgcctcaccatagacgatcttcaccacttataccattcctatctccagcacaacctcataaccatagccccactctttgccttcacggttttcggttcggttctctacatcgtaacccggcccaaaccggtttacctcgttgagtactcatgctaccttccaccaacgcattgtagatcaagtatctccaaggtcatggatatattttatcaagtaagaaaagctgatccttctcgtaacgggacgtgcgatgactcgtcgtggcttgacttcttgaggaaaattcaagaacgttcaggtctaggtgatgaaacacatggacccgagggactgcttcaggtccctccccggaaaacttttgcggcggcgcgtgaagagacggagaaagtaatcatcggtgcgctcgaaaatctattcgaaaacaccaaggttaaccctaaagatataggtatacttgtggtgaactcaagcatgtttaatccaactccttccctatccgccatggttgttaatactttcaagcttcgaagtaacgtaagaagctttaatcttggtggcatgggctgtagtgctggtgttatagccattgatctggctaaggacttgttgcatgtccataaaaacacgtatgctcttgtggtgagcacagagaacatcacttataacatttatgctggtgacaatagatcaatgatggtttcaaactgcttgttccgtgttggtggggcggccattttgctctccaacaagcctagagatcgtagacggtccaagtacgagttagttcacacggtccgaacgcataccggagctgacgacaagtcttttcgttgcgtgcaacaagaagacgatgagagcggcaaaaccggagtgagtttgtccaaggacataaccgatgttgctgggagaacggttaagaagaacatagcaacgttgggtccgttgattcttcctttaagcgagaaacttctttttttcgtgaccttcatggccaagaaacttttcaaagataaagttaagcattactacgtcccggatttcaagcttgctattgaccatttttgtatacatgctggagggagagccgtgatcgatgtgctagagaagaacctaggcctagcaccgatcgatgtggaggcatcaagatcaacgttacatagatttggtaacacttcatctagctcaatatggtatgaattagcatacatagaagcaaaaggaaggatgaagaaaggtaataaagtttggcaaattgctttaggatcagggtttaagtgtaacagtgcggtttgggtggctctaaacaatgtcaaggcttcgacaaatagtccttgggaacattgcatcgacagatatccggttaatattgattctgattcagctaagtcagagactcgtgtccaaaacggtcggtcctaa

SEQ ID NO: 10 - DNA, 1521 bp, Cardamine graeca
atgacgtccattaacgtaaagctcctttaccattacgtccttaccaactttttcaacctctgtttgttcccgttaacggcgttccctgccggaaaagcctctcagcttactacaaacgatctccaccacttatattcctatctccaccacaaccttataaccgttactctactctttgctttcaccgttttcggttcgattctctacatcgtaacccgacccaaaccggtttacctcgttgactattcctgctaccttcctccacgtcatctcagttgtggtatctctagggtaatggaaattttctatgaaataaggaaatctgatccttctcgcgaggtgccatttgatgatccgtcttcgcttgaattcttgaggaagattcaagaacgttcaggtctaggtgatgaaacctacggtcctcaaggactcgttcatgatatgccactacggatgaattttgcggcggcacgtgaagagacagagcaagtaatcaacggtgcgctcgaaaaactattcgagaacaccaaagttaaccctagagagattggtatacttgtggtgaattcaagcatgtttaatccaactccttcgctgtcggcgatggtcgttaatacattcaagctccgaagcaacatcaagagctttagtcttgggggcatgggttgtagtgctggtattatcgccattgatcttgctaaagacttgttgcatgttcacaaaaacacttatgctcttgtggttagcacagagaacatcactcacagcacttatactggtgataatagatccatgatggtttcaaattgcttgttccgtatgggtggggccgcgattttgctctctaacaaggcgggagatcgaagacggtccaagtacaagctagctcacacggttcgaacgcataccggagccgacgatcagtcttttcgatgtgttcgtcaagaagacgatgatagaggaaaaatcggagtttgtttgtccaaggacataacagctgttgcagggaaaacggttacgaaaaacatagcaacattgggtccgttggttcttcctttgagcgaaaagtttctttatgtcgtttccttgatggccaagaaacttttcaagaacaagatcaagcacacttacgtcccggatttcaaacttgctattgaccatttttgtatccatgctggaggcagagccgtgatcgacgtgcttgagaagaacttagcgctatcaccggttgacgtggaggcatcaagatcaacgttacatagatttgggaatacttcgtctagctcaatttggtatgaattggcatacatagaggcaaaaggaaggatgaagaaagggaataaagtttggcagatagctatagggtcagggtttaagtgtaatagtgcggtttgggtggctctatgcaatgtcaagccttcggtaaacagtccatgggaacattgcatcgatagatatcctgttgagattaactatggttcgtcaaagtcagagactcgtgcccaaaacggtcggtcctaa

SEQ ID NO: 11 - DNA, 1518 bp, Lunaria annua
atgacgtccattaacgtaaagctcctttaccattacgtcataaccaactttttcaacctctgtttcttcccactgacggcgatcctcgccggaaaagcctctcgtcttaccacaaacgatctccaccacttctattcatatctccaacacaaccttataaccttaaccctactctttgccttcaccgtttttggttcggttctctacttcgtaacccgacccaaaccggtttacctcgttgactactcctgctaccttccaccacaacatcttagcgctggtatctctaagaccatggaaatcttttatcaaataagaaaatctgatcctttacgaaacgtggcattagatgattcgtcttctcttgatttcttgagaaagattcaagagcgttcaggtctaggcgatgaaacctacggccccgagggactgtttgagattcctccgaggaagaatttagcgtcggcgcgtgaagagacggagcaagtaatcaacggtgcgctaaaaaatctattcgagaacaccaaagttaaccctaaagagattggtatacttgtggtgaactcaagcatgtttaatccgactccttcgttatccgcgatggtagttaatactttcaagctccgaagcaacatcaaaagctttaatcttggaggaatgggttgcagtgctggtgttatcgccattgatctagctaaagacttgttgcatgttcataaaaacacatatgctcttgtggtgagcacagagaacatcactcaaaacatttataccggtgataacagatccatgatggtttcgaattgcttgttccgtgtcggtggggcagcgattctgctctccaacaagccgggggatcgaagacggtccaagtacaggctagctcacacggttcgaacgcataccggagctgacgacaagtcttttggatgtgtgcggcaagaagaagatgatagcggtaaaaccggagttagtttgtcaaaagacataaccggtgttgccgggataacggttcagaaaaacataacaacattgggtccgttggttcttcctctgagcgaaaaaatcctttttgtcgttacattcgtagccaagaaactattaaaagataagatcaaacactattacgtgccggatttcaaacttgcagtagatcatttctgtattcatgcgggaggtagagccgtgatagatgtgttagagaagaacttagggctatcgccgatagatgtggaggcatcaagatcaacattacatagatttgggaatacatcgtctagttcaatttggtatgaattagcatacatagaggcaaaaggaaggatgaagaaaggtaataaagcttggcaaatagctgttgggtcaggttttaagtgtaatagtgcggtttgggtcgctttacgcaatgtcaaggcttcagctaatagtccttgggaacattgcattcacaaatatccggttcagatgtattctggttcatcaaagtcagagactcgtgcccaaaacggtcggtcctaa

SEQ ID NO: 12 - DNA, 1239 bp, artificial sequence
  Yarrowia lipolytica 26S rDNA
ttcacctccttcatccgagattacccgctgaacttaagcatatcaataagcggaggaaaagaaaccaacagggattgcctcagtaacggcgagtgaagcggcaaaagctcaaatttgaaaccctcgggattgtaatttgaagatttggcattggagaaagctaacccaagttgcttggaatagtacgtcatagagggtgacaaccccgtctggctaaccgttctccatgtattgccttatcaaagagtcgagttgtttgggaatgcagctcaaagtgggtggtaaactccatctaaagctaaatactggtgagagaccgatagcgaacaagtactgtgaaggaaaggtgaaaagaactttgaaaagagagtgaaatagtatgtgaaattgttgatagggaaggaaatgagtggagagtggccgaggtttcagccgcccctcgtgggcggtgtactgccgacgccgagtcatcgatagcgagacgagggttacaaatgggagcgccttcgggcgttctcccctaaccctccacactgccaccgacgacataatccacccatttcacccgtcttgaaacacggaccaaggagtctaatggatatgtgagtgttagggtggcaaaccccagcgcgcaatgaaagtgaatggattcgttcagaatcgaccgaacttgattattatgacagttttgagtaaacacatccattgggacccgaaagatggtgaactatgcctggatagggtgaagtcagaggaaactctgatggaggctcgtagcggttctgacgtgcaaatcgatcgtaggatctgggtataggggcgaaagactaatcgaaccatctagtagctggttcctgccgaagtttccctcaggatagcagaagctcatatcagttttatgaggtaaagcgaatgattagaagtattgggggcgaaatgccctcggcttattctcaaactttaaatatgtaagaagccttggttacttaatcgaaccgtggctacgaatgaagagcttctagtgggccatttttggtaagcagaactggcgatgcgggatgaaccgaacgtggagttaaggtgccggaatacacgctcatcagacaccacaaaaggtgttagtttatctagacagccggacggtggccatggaagtcggaatccgctaaggagtgtgtcacaactcaccggccgaatgaactagccctgaaaatggatggcgcttaagcgtgttaccta

SEQ ID NO: 13 - DNA, 1390 bp, artificial sequence
  Yarrowia lipolytica 26S rDNA
tagtgcagatcttggtggtagtagcaaatattcaaatgagaactttgaagactgaagtggggaaaggttccgtgtgaacagcagttggacacgggtaagtcgatcctaaggggtggcataactgtcgcgtacggcccgataagggccttctccaaaagggaagccggttgaaattccggcacttggatgtggattctccacggcaacgtaactgaatgtggggacggtggcacaagtcttggaaggagttatcttttctttttaacggagtcaacaccctggaattagtttgtctagagatagggtatcgttccggaagaggggggcagctttgtcccctccgatgcacttgtgacgccccttgaaaacccgcaggaaggaatagttttcacgccaagtcgtactgataaccgcagcaggtctccaaggtgaacagcctctagttgatagaataatgtagataagggaagtcggcaaaatagatccgtaacttcgggataaggattggctctgggggttggtggatggaagcgtgggagaccccaagggactggcggctgggcaactggcagccggacccgcggcagacactgcgtcgctccgtccacatcatcaaccgccccagaactggtacggacaaggggaatctgactgtctaattaaaacatagctttgcgatggttgtaaaacaatgttgacgcaaagtgatttctgcccagtgctctgaatgtcaaagtgaagaaattcaaccaagcgcgcgggtaaacggcgggagtaactatgctctcttaaggtagccaaatgcctcgtcatctaattagtgacgcgcatgaatggattaacgagattcccactgtccctatctactatgtagcgaaaccacagccaagggaacgggcttggcagaatcagcggggaaagaagaccctgttgagcttgactctagtttgacattgtgaagagacatagggggtgtagaataagtgggagcttcggcgccggtgaaataccactacccttatcgtttctttacttatttagtaagtggaagtggtttaacaaccattttctagcattcctttccaggctgaagacattgtcaggtggggagtttggctggggcggcacatctgttaaaagataacgcagatgtcctaagggggactcaatgagaacagaaatctcatgtagaacaaaagggtaaaagtccccttgattttgattttcagtgtgaatacaaaccatgaaagtgtggcctatcgatcctttagttgttcggagtttgaacctagaggtgccagaaaagttaccacagggataactggcttgtggcagtcaagcgttcatagcgacattgctttttgatccttcgatgtcggctcttcctatc

SEQ ID NO: 14 - DNA, 1033 bp, artificial sequence
  the Yarrowia lipolytica FAD2 gene
ggcagggtttgttggtgttaatgtgaacacagctttttttttgcttaataagatctccaaacacgttcaaaaaacacccactagttaaaagctcagttggactacctattgttccttctaatatacagtagactgctcgtacagtagtctctctaatcgatcggtgtctcaatgtctcaccgttaccggatacgcttatggtcgattgaattgccaatggaattatcggtggaaattcatggaaaaccggtttcggcgagctcgaaatacaccccgctatcgtacaagtcgaacgaatatcaggcgcccagacagatcgattcaagtagggagaagagtggaacaacttgtaaagaatgactgatggtgacgctcgggcccaggctagcactgaccatcaaatccatcttatcgatctgcttgaatctacaagtaggagggttggagtgattaagtgaaacttctttaacggctctatgccagttctattgatatccgaaacatcagtatgaaggtctgataagggtgacttcttcccacagattcgtatcagtacgagtacgagtaccggtacttgtaacagtattgatactaaagggaaactacaacggttgtcagcgtaatgtgacttcgcccatgaacgcagacacgcagtgccgagtgcggtgatatcgcctactcgttacgtccatggactacacaacccctcggcttcgcttggcttagcctcgggctcggtgctgttcagttaaaacacaatcaaataacatttctagctctactttttagaaggcaggccgtcaggagcaactccgactccattgacgtttctaaacatctgaatgccttccttaccttcaacaaactggcaggttcgggcgacagtgtaaagagacttgatgaagttggtgtcgtcgtgtcggtagtgcttgcccatgaccttcttgatcttctcagtggcgattcgggcgttgtagaagggaattcgagacacgtagtggtgcagaacgtgggtctcgatgatgtcatggaa

SEQ ID NO: 15 - DNA, 1046 bp, artificial sequence
  the Yarrowia lipolytica FAD2 gene
agtgaactcgttgccaaaggtgtcgtagacgggctcggacaccttctcaatgggcttaatgaaggccgtggggggctgcacggccaccttgccggtgccggtgttggtctgcgtggtcgaatccatttctatggtcggtctgttggaatacgagaaagggactcaggatgccgaccggtatatatttcaatgtcttacctcgagtttaaacccactaggcttttttttttctccctgtcaatccaccaacctttttggcctggcgtgactgacttggggacaagcaaaagctgagggtaaacagaggcacacccgaggttatatgttgagggccaatgtcaaattttcctcctaatcctgagagcccctctaacaccagcacgcatctacctcttgtatataactacgggccccgcctctcctaaccgccactttaacacgctcgtactcctcgtctgttaccacctgaaaaacgcataatgcgcatgtgcggattggccaagagagctccgaacggaaccgcccggggtatactgctgctctcagcgtggatagtgtggagggaccacgtctcaaccgtgacatgggtcgacttatggcgggggggagagtgaaagaaccagttacacgtgcacgtgaagaggggaagaccttggacgtgttcacgtgactacgtcggttctacatgaatccaacgtctcttatttcgtcatgtgctactacatgacccccattggcacgactctctctctgtgctgccactacttgacgactatgtccgcttgttgactcgttgaacaggtgtccgatgaatagcatggcttctcaacaggccatgcttaaagttagagttgggagatgtcgttccgaaccttgtgggcggcggtgtggaaagatagagagtacaagacaaccaaactcttggagcctttggctcgtaaagagagctcttccggtccatcgacgaagaaacgcagcgttgaaagactgccagaagcggcagtcaccgccgtatctgagacattgatcgtacacactcttgcaca

SEQ ID NO: 16 - DNA, 23 bp, artificial sequence
  primer
atttcttaaccccacgttgccgg

SEQ ID NO: 17 - DNA, 30 bp, artificial sequence
  primer
ccagcatctgcggttagtactgcaaaaagt

SEQ ID NO: 18 - DNA, 28 bp, artificial sequence
  primer
accgcagatgctggaactgcaggagtgg

SEQ ID NO: 19 - DNA, 40 bp, artificial sequence
  primer
caacgtggggttaagaaatcagagaagccactttgggcac

SEQ ID NO: 20 - DNA, 23 bp, artificial sequence
  primer
agaagataaccccacgttgccgg

SEQ ID NO: 21 - DNA, 30 bp, artificial sequence
  primer
cggccatctgcggttagtactgcaaaaagt

SEQ ID NO: 22 - DNA, 23 bp, artificial sequence
  primer
ccgcagatggccgagcccaagct

SEQ ID NO: 23 - DNA, 32 bp, artificial sequence
  primer
aacgtggggttatcttctgccgccctgttccc

SEQ ID NO: 24 - DNA, 23 bp, artificial sequence
  primer
ccatttaaccccacgttgccggt

SEQ ID NO: 25 - DNA, 30 bp, artificial sequence
  primer
cagccatctgcggttagtactgcaaaaagt

SEQ ID NO: 26 - DNA, 25 bp, artificial sequence
  primer
accgcagatggctgagcccaagctg

SEQ ID NO: 27 - DNA, 34 bp, artificial sequence
  primer
aacgtggggttaaatggcagacactttgggcacg

SEQ ID NO: 28 - DNA, 20 bp, artificial sequence
  primer
cgcttaaccccacgttgccg

SEQ ID NO: 29 - DNA, 30 bp, artificial sequence
  primer
cgtgcatctgcggttagtactgcaaaaagt

SEQ ID NO: 30 - DNA, 24 bp, artificial sequence
  primer
ccgcagatgcacgccgccatctct

SEQ ID NO: 31 - DNA, 29 bp, artificial sequence
  primer
cgtggggttaagcggcggggatcataacg

SEQ ID NO: 32 - DNA, 20 bp, artificial sequence
  primer
tgtggttgggactttagcca

SEQ ID NO: 33 - DNA, 20 bp, artificial sequence
  primer
aataagagcctcgacctggg

SEQ ID NO: 34 - DNA, 22 bp, artificial sequence
  primer
tgtgacttgcagatgtgaatca

SEQ ID NO: 35 - DNA, 20 bp, artificial sequence
  primer
cttaacggcaagtgtgggaa

SEQ ID NO: 36 - DNA, 21 bp, artificial sequence
  primer
caccttgtactgacagtcaca

SEQ ID NO: 37 - DNA, 20 bp, artificial sequence
  primer
caacaagtccatcagtaggg

SEQ ID NO: 38 - DNA, 1566 bp, Malania oleifera
atggacggctcttcgcaaatcaaggagctttcatgtcttgtgaaatttgtagaagaaactgtgaggatagagcatgcttcaaacccaaataagccagtttatttggtaggggattcttttggtggatgcttggcacttgctgttgctgctcgtaatcctacatttgatctggttctgattttagtcaatccagcaacgtcatttggcaggtcacagctgcaacctctgctgcctgtcttagaggctttgccggatgggcttcatttcactgttccttatctccttagctttatcatgggtacgtgttctgctgctttgaagccttaccgtgatccactgaagttggcaatggtcaatattgaaactaggtttcctcctgcactagtactagagcaattgtctggcaacctcacagctttgctaccacgcctttctggcttggctaatattataccgaaggagactcttctttggaagctaaagctcctaaaatcagctgctgcttatgctaattcacgtctccatgctgttaaagctgaagtacttgttctggctagtggcagtgataacatgctacctagcaaagatgaagctgaacgcctttcacgttcattacagaattgcatagttcgtctctttaaggacaatgggcatacccttctattggaagatggctatagtctgctgaccatcattaaatgtacttccaaataccgttgttcaaggaagcatgatttcatcacggattttctgcctccaagtatgtctgaattcaaacaggaattgaaccagagatttgggttatttcgtgttgctactagtcccatactgttctcaacactaccagatgggaagatagttaaaggtcttgccggaatcccaaatgaaggtcccgtcttattagttggttaccacatgttgttgggatgtgaactaggtccacttgttgaagcattcttgaaagagaagaatattatgattcgcggtgtagcgcacccagagatgttttcaaagaagcatgaaggtccatcaaatgaatttggaccttttgatttggtgaaactgtttggtggccttcctgtcacaccaagaaaccttttcaaattgttttcaacaaaatcacatatactcctttatccaggaggtgcacgtgaggctcttcatcgcaagggcgaaaagtacaagttattgtggcccaaccagcctgaatttgttagaatggctgcaagatttggtgccaccattgtaccgtttgggactgttggagaagacgacatagcagaagcggaatcgactatgttggcaaagaagatcacgctgaggagctctgacggcgagacctttgaggttgacaagatcgtggctcttgagtctcagatgatcaagcacatgattgaggatgactgtgcggacaatggaatacccttgcccaacgtcaccagctggatcttggtgaaggtcatcgagtactgcaagaagcacgtcaaggctcccaagatcgagaaacgaggcgacgtcaacaaggagctcaagtcgtgggacgctgagtttgtcaaaattgactag

SEQ ID NO: 39 - protein, 521 aa, Malania oleifera
MDGSSQIKELSCLVKFVEETVRIEHASNPNKPVYLVGDSFGGCLALAVAARNPTFDLVLILVNPATSFGRSQLQPLLPVLEALPDGLHFTVPYLLSFIMGTCSAALKPYRDPLKLAMVNIETRFPPALVLEQLSGNLTALLPRLSGLANIIPKETLLWKLKLLKSAAAYANSRLHAVKAEVLVLASGSDNMLPSKDEAERLSRSLQNCIVRLFKDNGHTLLLEDGYSLLTIIKCTSKYRCSRKHDFITDFLPPSMSEFKQELNQRFGLFRVATSPILFSTLPDGKIVKGLAGIPNEGPVLLVGYHMLLGCELGPLVEAFLKEKNIMIRGVAHPEMFSKKHEGPSNEFGPFDLVKLFGGLPVTPRNLFKLFSTKSHILLYPGGAREALHRKGEKYKLLWPNQPEFVRMAARFGATIVPFGTVGEDDIAEAESTMLAKKITLRSSDGETFEVDKIVALESQMIKHMIEDDCADNGIPLPNVTSWILVKVIEYCKKHVKAPKIEKRGDVNKELKSWDAEFVKID

SEQ ID NO: 40 - DNA, 1209 bp, Malania oleifera
atggcggagaccgaggtcagagagtcgccgttgaccgccgcccctgcccccgaggtgactgtcatcgagagcccccgagttcccctgctccattccgtgctcgccaccgccctgtggattggttgcatccacctgttcttcgccgtcatgttcaccgccactttcctgctccccctctccaaatccattgcggtgtttgctctgctactggttcttattgtggttcctgttgaggctgatagtaaatttgggatgaaagtaaggaggggcaataaccatcatgataatgaaggtgatgatgaagagttctccaacatacatggttgggttgtaaaaaaaatggtggtggtttattgccacagtgtcactatgccagaactggaggtgacaatgctgccaagtaacggttctgttttgtccttcacagtctttgcgttggagccacattcagtgttgcctgttggtgtcatctcacttatgcacctttcaaatgctgtgcccctcccaaaaactagggttcttgccagtagcgctgtgtttagaacaccattcctgaggcatatatggacatggatgggccttgcagctgtaacaaggaaaaattttatctcccttttggcagctggttatagttgcgccataataccaggtgggacgagggagacattgcttatggtgcaagatcatgaggtttatctcttgaaactctctgtggctctattgcgtattgctgcacgctctacagctttggagtggaacttgtgcccattccagaagattgctttccttaagacgagaaaaggatttgttcgcacggctatagagaccggtgtgcctctaatccctgttttctctttcggccaggtatttttttttttttggaaagatcaagtttacaccgatgttcttctggggagttttgggatgctacatctcataacatggacagggctcctttccacacatcacacacgaatgccttctttcttcatcatgaggagagctgccactgttcccctaactcctatgcctcgtcggcttccattgcatgtggttgtgggtagaccaattgaggttaagcaaaattcacaacccacagcagaagaggtgaatgaagtgcacagtcagtttgtgggggcattgcaagatctgttcgagaggcacaaagcaagggttgggcacgctgatcgtgagctgaaaatcatttga

SEQ ID NO: 41 - protein, 402 aa, Malania oleifera
MAETEVRESPLTAAPAPEVTVIESPRVPLLHSVLATALWIGCIHLFFAVMFTATFLLPLSKSIAVFALLLVLIVVPVEADSKFGMKVRRGNNHHDNEGDDEEFSNIHGWVVKKMVVVYCHSVTMPELEVTMLPSNGSVLSFTVFALEPHSVLPVGVISLMHLSNAVPLPKTRVLASSAVFRTPFLRHIWTWMGLAAVTRKNFISLLAAGYSCAIIPGGTRETLLMVQDHEVYLLKLSVALLRIAARSTALEWNLCPFQKIAFLKTRKGFVRTAIETGVPLIPVFSFGQVFFFFWKDQVYTDVLLGSFGMLHLITWTGLLSTHHTRMPSFFIMRRAATVPLTPMPRRLPLHVVVGRPIEVKQNSQPTAEEVNEVHSQFVGALQDLFERHKARVGHADRELKII

SEQ ID NO: 42 - DNA, 819 bp, Malania oleifera
atggactttgtacccgacatctccgccatcaagaccgacaagattaaaattgacaaggaaaccaccgacatgcttaccgctcggcatgacggatcttctgaagttagggaggacgagttggtggctgcgccagtgccaacttctccgttcggttgttgggccggcggacccggtaggagcatcaaccgtcgcacaaatcaaatacctctcgaaccttgcagagacatctcagttcataaactaatcgaaccgatgtgctcaaaaagactagggagtgatttctccgaccagttagcgtcaccttgtgtgtctcattcgtggttgccggcgacgacgaagtgcgatcatgtgcactgcctgtgcatggaacgtgcctgctgctggaattggtcctctgatgatgtgctttcagctgctggcggatcaagtcgtgttgaatctaatagtgttcatggcgtattaagaaaactccagcaatggtctgcaatgaacagtgctgccgatggggggacaaaggggctggaatttgacagaaaagacacgaagaacaagaatgtgatgaaagagagtacagtgaccactccaaagaccttgagggttgcattgaaatgctgcacaagggaagatactgcaccggaggcaaaagagaatatgaattatttccgtggtatagaatgttgtgaggttaaggaggcatattcgaaggcactgcatgattctgttactgaacaatacaatgtgctcaaatctgccatacatggcaaacaaggactggaggcatccattccagatgtctcattatcacaaccatggcagtag

SEQ ID NO: 43 - protein, 402 aa, Malania oleifera; identical to SEQ ID NO: 41

SEQ ID NO: 44 - DNA, 1110 bp, Malania oleifera
atggtgctgtggcagtgcggtgggtctggactcagaggcagcgatgaaggtttgcgatggcacggcgctgctatgcttgcaactcgcacggtgccggcagcggcaggtctggacagtggacgccactcgcacaatgtccaaggtagccaacctcaaatccaggagatctgtgcgaaagagagcttggggaatattgacggtgtgaggggtgactctattaatgatgcggagtgggctggtaaggctgtgacctatgtagcaggggatcgggttttaacggatattctttgcaagcccttcagcatgggcagaaatcttatgtgcgtctactcaaaaaagcacatgcttgatgatcctaagcttgctgagatgaagaaaaaagcaaatatacgaagtttgaaagaaatggccatgcttttgagaggagggtcacaaatagtatggattgcaccaagtggtggtagggaccgtccagatccccagacaggagaatggcatccggcaccctttgatgcttcttcagtggacaatatgaggcggcttgcagaaaatgctggtgttcctgcacatatttatccattagcattaatttgctacaacattatgccgcctccacccaaggttgagaaagagattggagagaaaagagtggtatcctttcatggggttggactatccgtgataccagatataagctatgctgaaattgccgctgcttgtgaaaactctgaagagactggcgatgccgacacaaatcagtcacactaccaatgtcatcgcaggatcccgcaggcggagaaatttggcatcttggccgcattgcccgatgatgagtcaagggcgaaggccacatctcccagatctacgccatccaagcgccttcgttacaagatcgccggcttctccgcccacctcatgaagcgaatccagaagggtccctttcggggtatttctctgaagctgcaagaggaagagcacgagaggcgcatggacttcgtacccgacatctccgccatcaagaccgacaagattaaagtcgacaaggaaaccagatctacaccatccaggcgccttcgcaacaagatcgcgacttctccacccacctcatga

SEQ ID NO: 45 - protein, 369 aa, Malania oleifera
MVLWQCGGSGLRGSDEGLRWHGAAMLATRTVPAAAGLDSGRHSHNVQGSQPQIQEICAKESLGNIDGVRGDSINDAEWAGKAVTYVAGDRVLTDILCKPFSMGRNLMCVYSKKHMLDDPKLAEMKKKANIRSLKEMAMLLRGGSQIVWIAPSGGRDRPDPQTGEWHPAPFDASSVDNMRRLAENAGVPAHIYPLALICYNIMPPPPKVEKEIGEKRVVSFHGVGLSVIPDISYAEIAAACENSEETGDADTNQSHYQCHRRIPQAEKFGILAALPDDESRAKATSPRSTPSKRLRYKIAGFSAHLMKRIQKGPFRGISLKLQEEEHERRMDFVPDISAIKTDKIKVDKETRSTPSRRLRNKIATSPPTS

SEQ ID NO: 46 - DNA, 693 bp, Malania oleifera
atgcagctaagaatacttttagatgttttgactcttctgtttgcagcatttctttatttggaatctaatttggaggtattgttttcttgtcttgctgggtttcctgcagagctgctttctggaataaagaaggaaacagaagctggcagattgccttcaaattttgcttcagttctggttttccaaagtggaattccagatgctgatgaaattatattgtcaaacacaactgctttgtttgatcgtgttttactggatgcagaggactcttttgttttccccccacatcataaagcaatgcgagagccttttgattactacatgtttggtcaaaattatatccgtcctttgatagattttgggaattcatatgttggcaatatcaacatttttcatgaaatggaagagaagctgcagcaggtcaagaatctcaatgggattgagtggggtcagccatggaggagtctccactctctgcaaatagagagtaaatccttagatctgcgactggaaaaggttgggaagggtttctttttggctggatgctgttttcggttgcaaagggaaattgtcaagttaaattcttggatttggggttatactcatttggaaaggcttattctatttttgttctatggggttttgatggggagtgatggcaacggtttgttgagatgttgcagccgacggtaa

SEQ ID NO: 47 - protein, 230 aa, Malania oleifera
MQLRILLDVLTLLFAAFLYLESNLEVLFSCLAGFPAELLSGIKKETEAGRLPSNFASVLVFQSGIPDADEIILSNTTALFDRVLLDAEDSFVFPPHHKAMREPFDYYMFGQNYIRPLIDFGNSYVGNINIFHEMEEKLQQVKNLNGIEWGQPWRSLHSLQIESKSLDLRLEKVGKGFFLAGCCFRLQREIVKLNSWIWGYTHLERLILFLFYGVLMGSDGNGLLRCCSRR

SEQ ID NO: 48 - DNA, 1566 bp, Malania oleifera
atggacggctcttctcagatcaaggagctgtcttgcctggtgaagttcgtggaggagactgtgcgaatcgagcacgcctctaatcccaataagcccgtgtacctggtgggcgactctttcggcggatgtctggctctggctgtggctgctagaaatcctactttcgacctggtgctgatcctggtgaaccccgccacttctttcggcagatctcagctgcaacctctgctgcccgtgctggaggctctgcctgatggactgcatttcaccgtgccctacctgctgtctttcatcatgggcacctgctctgccgccctgaaaccctatagagatcccctgaaactggccatggtgaacatcgagactcgattcccccccgccctggtgctggaacaactttctggaaatctgaccgccctgctgcccagactgtctggactggctaatatcatccccaaggaaaccctgctgtggaagctgaagctgctgaagtctgccgccgcctatgctaattctcgactgcacgccgtgaaagccgaggtgctggtgctggcttctggatctgataacatgctgccctctaaggacgaggccgagcgactttctagatctctgcaaaattgcatcgtgcgactgttcaaggacaacggccacaccctgctgctggaggatggatattctctgctgaccatcatcaagtgcacctctaagtaccgatgctctcgaaagcacgacttcatcaccgacttcctgcccccctctatgtctgagttcaagcaggagctgaaccagcgattcggcctgttccgagtggccacttctcctattctgttttctaccctgcccgacggcaaaatcgtgaagggcctggctggaattcccaatgagggccctgtgctgctggtgggctatcatatgctgctgggatgtgagctgggccccctggttgaagcttttctgaaagagaaaaacatcatgatccgaggcgtggcccaccccgaaatgttttctaaaaagcacgagggcccctctaacgagttcggccctttcgatctggtgaagctgttcggcggactgcccgtgactcctagaaatctgtttaagctgttctctaccaagtcccacatcctgctgtaccccggcggcgctagagaagctttacatagaaaaggcgaaaagtacaagctgctgtggcccaaccagcccgagtttgtgagaatggctgctcgatttggcgccactatcgtgcctttcggaaccgtgggagaggacgacattgccgaggctgagtctaccatgctggctaagaaaatcaccctgcgatcttctgacggcgaaaccttcgaggtggacaagatcgtggccctggagtctcagatgatcaagcacatgatcgaggacgactgcgccgacaacggcattcctttacctaatgtgacctcttggatcctggtgaaggtgatcgagtactgcaagaagcacgtgaaggcccccaagatcgagaagcgaggcgatgtgaataaggagctgaagtcttgggacgccgagttcgtgaagatcgactaa

SEQ ID NO: 49 - protein, 1209 aa, Malania oleifera
ATGGCCGAGACTGAAGTGCGAGAGTCTCCCCTGACTGCCGCCCCTGCTCCTGAGGTGACTGTGATTGAATCTCCCAGAGTGCCCCTGCTGCACTCTGTGCTTGCTACTGCTCTGTGGATCGGCTGTATTCATCTGTTTTTCGCCGTGATGTTCACCGCCACCTTCCTGCTGCCTCTGTCTAAATCTATCGCCGTGTTCGCCCTGCTGCTGGTGCTGATTGTGGTGCCCGTTGAAGCCGATTCTAAGTTCGGCATGAAGGTGCGACGAGGCAACAACCACCACGACAACGAGGGCGATGACGAGGAGTTTTCTAACATCCACGGCTGGGTGGTGAAGAAGATGGTGGTGGTGTACTGCCACTCTGTGACCATGCCCGAGCTGGAGGTTACTATGCTGCCCTCTAATGGCTCTGTGCTGTCTTTCACCGTGTTCGCCCTGGAGCCCCACTCTGTGCTGCCTGTTGGAGTTATTTCTCTGATGCACCTGTCTAACGCCGTGCCCCTGCCTAAAACTAGAGTGCTGGCTTCTTCTGCCGTGTTCCGAACCCCTTTCCTGCGACATATCTGGACCTGGATGGGCCTGGCCGCTGTTACTAGAAAAAATTTCATCTCTCTGCTGGCCGCCGGCTACTCTTGCGCTATTATTCCCGGAGGAACTCGAGAAACCCTGCTGATGGTGCAAGACCACGAGGTGTACCTGCTGAAGCTGTCTGTGGCCCTGCTGCGAATTGCCGCTAGATCTACTGCCCTGGAATGGAACCTGTGTCCCTTTCAGAAAATCGCCTTCCTGAAGACCCGAAAGGGCTTCGTGCGAACCGCCATTGAAACCGGAGTGCCCCTTATTCCTGTGTTCTCTTTCGGCCAGGTGTTCTTCTTCTTCTGGAAGGACCAGGTGTACACCGACGTGCTGCTGGGCTCTTTTGGCATGCTGCACCTGATCACCTGGACCGGCTTACTGTCTACTCACCATACCCGAATGCCCTCTTTCTTCATCATGCGACGAGCCGCCACCGTGCCCCTTACTCCCATGCCTAGAAGACTGCCTCTGCATGTGGTGGTGGGACGACCTATTGAGGTGAAACAGAACTCTCAGCCCACCGCCGAGGAAGTGAATGAGGTGCATTCTCAGTTCGTGGGCGCCCTGCAAGATCTGTTCGAGCGACATAAGGCCAGAGTGGGCCACGCCGATAGAGAACTGAAAATCATTTAA

SEQ ID NO: 50 - DNA, 819 bp, Malania oleifera
atggacttcgtgcccgacatctctgccatcaagaccgacaagatcaagatcgacaaggagactaccgacatgctgaccgccagacatgatggctcttctgaggtgagagaagacgagctggtggccgcccctgtgcctacttctccttttggatgttgggctggcggacccggcagatctatcaacagaagaactaatcagatccccctggagccctgccgagacatttctgtgcataaactgatcgagcccatgtgctctaagcgactgggctctgacttctctgaccagctggcctctccctgcgtgtctcactcttggctgcctgctactaccaaatgcgaccatgtgcactgcctgtgcatggagcgagcctgttgttggaattggtcttctgacgacgtgctgtctgccgccggaggatcttctagagtggaatctaactctgtgcacggcgtgctgcgaaagctgcagcaatggtctgccatgaactctgccgccgatggaggcactaaaggactggagtttgatcgaaaggacaccaagaacaagaacgtgatgaaggagtctaccgtgaccacccccaagaccctgagagtggctctgaaatgctgtacccgagaggataccgcccccgaagctaaagagaacatgaactacttccgaggcatcgagtgctgcgaggtgaaggaggcttattctaaggccctgcacgactctgtgaccgagcagtataatgtgctgaagtctgccatccacggcaagcagggcctggaggcttctattcccgatgtgtctctgtctcagccctggcagtaa

SEQ ID NO: 51 - DNA, 1110 bp, Malania oleifera
atggtgctgtggcagtgcggaggatctggactgagaggatctgacgaaggactgcgatggcacggcgctgctatgttagctactagaactgtgcctgctgctgctggactggactctggaagacattctcataacgtgcagggctctcagccccagatccaagagatttgcgccaaggagtctctgggcaacatcgacggcgtgcgaggagattctattaacgacgccgaatgggccggcaaagccgtgacttatgtggctggcgatcgagtgctgaccgatattctgtgcaagcccttctctatgggccgaaacctgatgtgcgtgtactctaagaagcacatgctggacgaccccaagctggccgaaatgaagaagaaggccaacatccgatctctgaaggagatggccatgctgctgcgaggcggatctcaaatcgtgtggatcgccccctctggcggcagagatagacctgatcctcaaactggagagtggcaccccgctccctttgacgcttcttctgtggacaacatgcgacgactggccgagaacgccggagttcctgctcatatttatcctctggctctgatctgttacaacatcatgccccctccccccaaggtggaaaaagagattggagagaagcgagtggtgtctttccacggcgtgggcctttctgtgattcccgacatttcttacgccgagatcgccgccgcttgtgaaaactctgaagagactggagatgccgacaccaaccagtctcattatcagtgccaccgacgaatcccccaggctgaaaaatttggcattctggccgctctgcctgacgatgagtctcgagctaaagccacctctccccgatctaccccttctaaacgactgcgatacaagatcgccggcttctctgcccacctgatgaagcgaattcagaagggccccttccgaggcatttctctgaagctgcaggaggaggagcacgagcgacgaatggatttcgtgcccgacatttctgccatcaagaccgacaagatcaaggtggacaaggaaacccgatctaccccctctcgacgactgcgaaataagatcgccacctctccccccacctcttaa

SEQ ID NO: 52 - DNA, 693 bp, Malania oleifera
atgcagctgcgaatcctgctggacgtgctgaccttactgtttgccgcttttctgtacctggagtctaacctggaggtgctgttctcttgcctggccggctttcctgctgaactgctgtctggaattaagaaggagactgaggccggccgactgccctctaattttgcatctgtgctggtgttccagtctggcatccccgacgctgatgaaatcattctgtctaacaccaccgccctgttcgaccgagtgctgcttgatgctgaagactctttcgtgttccccccccaccacaaggccatgagagaaccttttgattactacatgttcggccagaactacatccgacccctgatcgacttcggcaactcttacgtgggcaacatcaacatcttccacgagatggaggagaagctgcagcaggtgaagaacctgaacggcatcgagtggggccagccctggagatctctgcattctctgcagatcgagtctaagtctctggacctgcgactggagaaggtgggcaaaggatttttcctggccggatgctgttttcgactgcagcgagagatcgtgaagctgaactcttggatctggggctacacccacctggagcgactgatcctttttctgttctacggcgtgctgatgggctctgacggcaatggactgctgagatgttgctctcgacgataa